European Patent Specification EP 3 834 822 B1, published October 25, 2023. Title: Polymeric nanoparticle composition for delivering oncolytic virus and preparation method thereof. Applicant: SAMYANG BIOPHARMACEUTICALS CORPORATION. The sequence listing filed with the application follows.

SEQUENCE LISTING (1 sequence)

SEQ ID NO: 1 - DNA, 1646 bp, Artificial Sequence
  Firefly Luciferase
atgccaaaaacattaagaagggcccagcgccattctacccactcgaagacgggaccgccggcgagcagctgcacaaagccatgaagcgctacgccctggtgcccggcaccatcgcctttaccgacgcacatatcgaggtggacattacctacgccgagtacttcgagatgagcgttcggctggcagaagctatgaagcgctatgggctgaatacaaaccatcggatcgtggtgtgcagcgagaatagcttgcagttcttcatgcccgtgttgggtgccctgttcatcggtgtggctgtggccccagctaacgacatctacaacgagcgcgagctgctgaacagcatgggcatcagccagcccaccgtcgtattcgtgagcaagaaagggctgcaaaagatcctcaacgtgcaaaagaagctaccgatcatacaaaagatcatcatcatggatagcaagaccgactaccagggcttccaaagcatgtacaccttcgtgacttcccatttgccacccggcttcaacgagtacgacttcgtgcccgagagcttcgaccgggacaaaaccatcgccctgatcatgaacagtagtggcagtaccggattgcccaagggcgtagccctaccgcaccgcaccgcttgtgtccgattcagtcatgcccgcgaccccatcttcggcaaccagatcatccccgacaccgctatcctcagcgtggtgccatttcaccacggcttcggcatgttcaccacgctgggctacttgatctgcggctttcgggtcgtgctcatgtaccgcttcgaggaggagctattcttgcgcagcttgcaagactataagattcaatctgccctgctggtgcccacactatttagcttcttcgctaagagcactctcatcgacaagtacgacctaagcaacttgcacgagatcgccagcggcggggcgccgctcagcaaggaggtaggtgaggccgtggccaaacgcttccacctaccaggcatccgccagggctacggcctgacagaaacaaccagcgccattctgatcacccccgaaggggacgacaagcctggcgcagtaggcaaggtggtgcccttcttcgaggctaaggtggtggacttggacaccggtaagacactgggtgtgaaccagcgcggcgagctgtgcgtccgtggccccatgatcatgagcggctacgttaacaaccccgaggctacaaacgctctcatcgacaaggacggctggctgcacagcggcgacatcgcctactgggacgaggacgagcacttcttcatcgtggaccggctgaagagcctgatcaaatacaagggctaccaggtagccccagccgaactggagagcatcctgctgcaacaccccaacatcttcgacgccggggtcgccggcctgcccgacgacgatgccggcgagctgcccgccgcagtcgtcgtgctggaacacggtaaaaccatgaccgagaaggagatcgtggactatgtggccagccaggttacaaccgccaagaagctgcgcggtggtgttgtgttcgtggacgaggtgcctaaaggactgaccggcaagttggacgcccgcaagatccgcgagattctcattaaggccaagaagggcggcaagatcgccgtgtaa